European Patent Application EP 4 785 964 A1, published August 5, 2026. Title: A pharmaceutical composition for preventing or treating cancer comprising nucleic acid construct encoding p53 protein. Applicant: HANMI PHARM. CO., LTD. The sequence listing filed with the application follows.

SEQUENCE LISTING (27 sequences)

SEQ ID NO: 1 - RNA, 50 nt, synthetic construct
  source 1..50: mol_type = other RNA
agccgtcttccatcgttacagtcaccgttttcgcattctgtctagccacc

SEQ ID NO: 2 - RNA, 50 nt, synthetic construct
  source 1..50: mol_type = other RNA
agaatccagtcaacgcatatccacgtatacccgaacacatcacagccacc

SEQ ID NO: 3 - RNA, 50 nt, synthetic construct
  source 1..50: mol_type = other RNA
agccccccaacactgacttaatcgctttaagttcctccaaacgagccacc

SEQ ID NO: 4 - RNA, 50 nt, synthetic construct
  source 1..50: mol_type = other RNA
agagcagaacgcgtaaccacaccatcgcaacatcccacttgatagccacc

SEQ ID NO: 5 - RNA, 70 nt, synthetic construct
  source 1..70: mol_type = other RNA
agaccagacacctaacagactagacattttaccgaaatccgcattaaccattctaactcgtatagccacc

SEQ ID NO: 6 - RNA, 70 nt, synthetic construct
  source 1..70: mol_type = other RNA
agatcactaacaccatataacgctatcttcctccttctccgacattccagtactcattccacaagccacc

SEQ ID NO: 7 - RNA, 70 nt, synthetic construct
  source 1..70: mol_type = other RNA
agtacccactccagataaactgacaaccatacgcgaacaacgacgaatcgtatcacacgcagaagccacc

SEQ ID NO: 8 - RNA, 70 nt, synthetic construct
  source 1..70: mol_type = other RNA
agcgagataacttacaaggagagagaagacgaggagagataaattagagagaaaacgagtaagagccacc

SEQ ID NO: 9 - RNA, 70 nt, synthetic construct
  source 1..70: mol_type = other RNA
agtaaactaaccactccatcacgtatatattcctctttcacacctttccattctcgaactaaccgccacc

SEQ ID NO: 10 - RNA, 178 nt, synthetic construct
  source 1..178: mol_type = other RNA
accaccaagacaaaaaccacgaatttacgccaaaagtggagtaaggaggtgcgtcccttacgcaacacgacagccgggatctaacaatagggttaatggactggttgagataaggggcattaaaaccaaacggtctacacataaaacgaatgaaaacttcctaaaggatcgacggtgg

SEQ ID NO: 11 - RNA, 178 nt, synthetic construct
  source 1..178: mol_type = other RNA
cataccataaaaccaaacatatacccgaggtccttcggcattgggaggatgatacgcaagaagcatgattccccaccagaccgaatgcaggtttaagtgaggggtgcaaacttgtgtcactaaccattattatgaagaaaaaaacagccaaaaaaagagccacaaggcggcgcggtat

SEQ ID NO: 12 - RNA, 178 nt, synthetic construct
  source 1..178: mol_type = other RNA
gccgctaaataaacgaacacgtacctacgctttgacaggagtgggcaagtgggaaggttaccggaactacgaggaccaccaggcaagtattggttagtcactcttccaactaatcttaataaaacgagacatcgaaaaaaaaaaaaggcaaaaacaagtccagaaggagccagggtgg

SEQ ID NO: 13 - RNA, 178 nt, synthetic construct
  source 1..178: mol_type = other RNA
agagtaaaattaatatacggtatagaactcaccattgtgcgttctacctcgaggtgtcatgacgacagtgtcccatatcaacccgagaagttggaaatgcggagtcgaacgtgacgccaataaggccaaaaggtaaataatgaaacgtacaaccgaatgccaaaaggctacgctgctc

SEQ ID NO: 14 - RNA, 178 nt, synthetic construct
  source 1..178: mol_type = other RNA
gtacatgctacaaaccatgcggaacctacaagacactttatgggtaaagcaacaaacccacttgtaaagttaccacaccggtcccatctgccggccgtgagtatatgatctgggtttataatctcgaaatatcgcgaaacaatatgcccttagaataagcacccatgcgggcaatgta

SEQ ID NO: 15 - RNA, 158 nt, synthetic construct
  source 1..158: mol_type = other RNA
tctttatgagaattactcattctgatttttaacatagcattttttttctgttgtgtagatgggccaaaggacattccataacttttcataaggacaaacgattaccgacggattggtactagttgttaattaacatctgggggatgtaaacatttttt

SEQ ID NO: 16 - RNA, 158 nt, synthetic construct
  source 1..158: mol_type = other RNA
tacgaactgaaataatcaagtgatagttatcaattaaaagctttataattttagtttccttgggccacggaatttccacaatttttagttcgtaaaccggtcatccaatctattgggttgaggctggaatatgcaccttatgggtgtctttgtataaa

SEQ ID NO: 17 - RNA, 158 nt, synthetic construct
  source 1..158: mol_type = other RNA
aacacagaaaactaccactatacttctatttagaaagcacttattaattgctttttgttagtgaaacatgcaaggcacccatgttttctgtgttaaccaagccagttgatattagctgtatgcttggattctatacataaaatgtatttaagcagctc

SEQ ID NO: 18 - RNA, 178 nt, Homo sapiens
  source 1..178: mol_type = mRNA
ccacacccccattcccccactccagataaagcttcagttatatctcacgtgtctggagttctttgccaagagggagaggctgaaatccccagccgcctcacctgcagctcagctccatcctacttgaaacctcacctgttcccaccgcattttctcctggcgttcgcctgctagtgtg

SEQ ID NO: 19 - RNA, 158 nt, Homo sapiens
  source 1..158: mol_type = mRNA
gtgtgtggaggacaccctgaaccccccgctttcaaacaagttttcaaattgtttgaggtcaggatttctcaaactgattcctttctttgcatatgagtatttgaaaataaatattttcccagaatataaataaatcatcacatgattattttaactat

SEQ ID NO: 20 - DNA, 17 bp, synthetic construct
  source 1..17: mol_type = other DNA
taatacgactcactata

SEQ ID NO: 21 - DNA, 61 bp, Homo sapiens
  source 1..61: mol_type = genomic DNA
agtgctccccatccaactaaactgtccctctgtccgaactaaactgcactgtcccagcacc

SEQ ID NO: 22 - DNA, 1179 bp, Homo sapiens
  source 1..1179: mol_type = genomic DNA
atggaagaacctcagtccgatccgagcgtcgagcctcccctgtcacaggaaactttcagtgacctgtggaaactgctgcccgagaataatgtactttcgcctctgcctagccaagcaatggatgatctgatgctgtctccagatgacatcgaacagtggtttacagaggatccagggcccgatgaggcaccacgaatgccagaggcggccccacctgttgcacccgcacctgcggctccaacacccgcagcccccgcccccgctccaagctggcctctcagtagttccgtgccatcacagaagacctatcaaggcagctacggatttcgcctcggatttctccattcaggcactgccaagtccgtgacttgtacgtacagccccgctctgaacaaaatgttctgtcagttggcgaagacatgtcctgtccagctttgggtagattctacccccccgccggggacacgggtgcgagccatggccatttataaacagtctcagcacatgaccgaggtcgtgcgcaggtgtcctcaccatgaacgatgctccgactccgacggcctggcccccccacagcacctgattcgcgtggaaggcaatcttcgtgtggagtacctcgatgatcggaacaccttcagacatagcgtggttgtgccttatgagccacccgaagttggaagcgactgtaccaccatccattacaactatatgtgcaacagtagctgcatgggtggcatgaatcggcggcctatcttgacaataatcactttagaggactcttccggaaacctgcttggcagaaattcattcgaggtccgtgtctgcgcctgcccgggcagggaccgcagaaccgaagaggagaatttacggaaaaagggggaaccccaccacgaactgccaccgggcagtaccaaaagggctctccctaataacacatcttcatcgccccagccaaagaagaaacccctcgacggagagtactttactctacaaattagggggagagaaagatttgagatgttccgcgaattgaacgaggccctggagttgaaagacgctcaagccggaaaggaaccaggtgggtctagggcccactcaagccatctgaagagtaagaaaggccagtccacttccaggcacaaaaagttaatgttcaagacggagggtcctgactctgac

SEQ ID NO: 23 - DNA, 158 bp, Homo sapiens
  source 1..158: mol_type = genomic DNA
gtgtgtggaggacaccctgaaccccccgctttcaaacaagttttcaaattgtttgaggtcaggatttctcaaactgattcctttctttgcatatgagtatttgaaaataaatattttcccagaatataaataaatcatcacatgattattttaactat

SEQ ID NO: 24 - DNA, 120 bp, Homo sapiens
  source 1..120: mol_type = genomic DNA
aaaaaaaaaaaaaaaaaaaaaaaaaaaaaaaaaaaaaaaaaaaaaaaaaaaaaaaaaaaaaaaaaaaaaaaaaaaaaaaaaaaaaaaaaaaaaaaaaaaaaaaaaaaaaaaaaaaaaaaa

SEQ ID NO: 25 - protein, 393 aa, Homo sapiens [sequence omitted]

SEQ ID NO: 26 - RNA, 61 nt, Homo sapiens
  source 1..61: mol_type = mRNA
agtcctccccatcctctccctctgtccctctgtccctctgaccctgcactgtcccagcacc

SEQ ID NO: 27 - RNA, 1558 nt, synthetic construct
  source 1..1558: mol_type = other RNA
agatcactaacaccatataacgctatcttcctccttctccgacattccagtactcattccacaagccaccatggaagaacctcagtccgatccgagcgtcgagcctcccctgtcacaggaaactttcagtgacctgtggaaactgctgcccgagaataatgtactttcgcctctgcctagccaagcaatggatgatctgatgctgtctccagatgacatcgaacagtggtttacagaggatccagggcccgatgaggcaccacgaatgccagaggcggccccacctgttgcacccgcacctgcggctccaacacccgcagcccccgcccccgctccaagctggcctctcagtagttccgtgccatcacagaagacctatcaaggcagctacggatttcgcctcggatttctccattcaggcactgccaagtccgtgacttgtacgtacagccccgctctgaacaaaatgttctgtcagttggcgaagacatgtcctgtccagctttgggtagattctacccccccgccggggacacgggtgcgagccatggccatttataaacagtctcagcacatgaccgaggtcgtgcgcaggtgtcctcaccatgaacgatgctccgactccgacggcctggcccccccacagcacctgattcgcgtggaaggcaatcttcgtgtggagtacctcgatgatcggaacaccttcagacatagcgtggttgtgccttatgagccacccgaagttggaagcgactgtaccaccatccattacaactatatgtgcaacagtagctgcatgggtggcatgaatcggcggcctatcttgacaataatcactttagaggactcttccggaaacctgcttggcagaaattcattcgaggtccgtgtctgcgcctgcccgggcagggaccgcagaaccgaagaggagaatttacggaaaaagggggaaccccaccacgaactgccaccgggcagtaccaaaagggctctccctaataacacatcttcatcgccccagccaaagaagaaacccctcgacggagagtactttactctacaaattagggggagagaaagatttgagatgttccgcgaattgaacgaggccctggagttgaaagacgctcaagccggaaaggaaccaggtgggtctagggcccactcaagccatctgaagagtaagaaaggccagtccacttccaggcacaaaaagttaatgttcaagacggagggtcctgactctgactgatgactcgagcataccataaaaccaaacatatacccgaggtccttcggcattgggaggatgatacgcaagaagcatgattccccaccagaccgaatgcaggtttaagtgaggggtgcaaacttgtgtcactaaccattattatgaagaaaaaaacagccaaaaaaagagccacaaggcggcgcggtatgctagcaaaaaaaaaaaaaaaaaaaaaaaaaaaaaaaaaaaaaaaaaaaaaaaaaaaaaaaaaaaaaaaaaaaaaaaaaaaaaaaaaaaaaaaaaaaaaaaaaaaaagaagagcgaatt